European Patent Specification EP 4 351 623 B1, published August 5, 2026. Title: GENE COMBINATION AS A BROAD SPECTRUM ANTIVIRAL. Applicant: Icahn School of Medicine at Mount Sinai. The sequence listing filed with the application follows.

SEQUENCE LISTING (11 sequences)

SEQ ID NO: 1 - DNA, 2148 bp, Homo sapiens
atgtctaaggcccacaagccttggccctaccggaggagaagtcaattttcttctcgaaaatacctgaaaaaagaaatgaattccttccagcaacagccaccgccattcggcacagtgccaccacaaatgatgtttcctccaaactggcagggggcagagaaggacgctgctttcctcgccaaggacttcaactttctcactttgaacaatcagccaccaccaggaaacaggagccaaccaagggcaatggggcccgagaacaacctgtacagccagtacgagcagaaggtgcgcccctgcattgacctcatcgactccctgcgggctctgggtgtggagcaggacctggccctgccagccatcgccgtcatcggggaccagagctcgggcaagagctctgtgctggaggcactgtcaggagtcgcgcttcccagaggcagcggaatcgtaaccaggtgtccgctggtgctgaaactgaaaaagcagccctgtgaggcatgggccggaaggatcagctaccggaacaccgagctagagcttcaggaccctggccaggtggagaaagagatacacaaagcccagaacgtcatggccgggaatggccggggcatcagccatgagctcatcagcctggagatcacctcccctgaggttccagacctgaccatcattgaccttcccggcatcaccagggtggctgtggacaaccagccccgagacatcggactgcagatcaaggctctcatcaagaagtacatccagaggcagcagacgatcaacttggtggtggttccctgtaacgtggacattgccaccacggaggcgctgagcatggcccatgaggtggacccggaaggggacaggaccatcggtatcctgaccaaaccagatctaatggacaggggcactgagaaaagcgtcatgaatgtggtgcggaacctcacgtaccccctcaagaagggctacatgattgtgaagtgccggggccagcaggagatcacaaacaggctgagcttggcagaggcaaccaagaaagaaattacattctttcaaacacatccatatttcagagttctcctggaggaggggtcagccacggttccccgactggcagaaagacttaccactgaactcatcatgcatatccaaaaatcgctcccgttgttagaaggacaaataagggagagccaccagaaggcgaccgaggagctgcggcgttgcggggctgacatccccagccaggaggccgacaagatgttctttctaattgagaaaatcaagatgtttaatcaggacatcgaaaagttagtagaaggagaagaagttgtaagggagaatgagacccgtttatacaacaaaatcagagaggattttaaaaactgggtaggcatacttgcaactaatacccaaaaagttaaaaatattatccacgaagaagttgaaaaatatgaaaagcagtatcgaggcaaggagcttctgggatttgtcaactacaagacatttgagatcatcgtgcatcagtacatccagcagctggtggagcccgcccttagcatgctccagaaagccatggaaattatccagcaagctttcattaacgtggccaaaaaacattttggcgaatttttcaaccttaaccaaactgttcagagcacgattgaagacataaaagtgaaacacacagcaaaggcagaaaacatgatccaacttcagttcagaatggagcagatggttttttgtcaagatcagatttacagtgttgttctgaagaaagtccgagaagagatttttaaccctctggggacgccttcacagaatatgaagttgaactctcattttcccagtaatgagtcttcggtttcctcctttactgaaataggcatccacctgaatgcctacttcttggaaaccagcaaacgtctcgccaaccagatcccatttataattcagtattttatgctccgagagaatggtgactccttgcagaaagccatgatgcagatactacaggaaaaaaatcgctattcctggctgcttcaagagcagagtgagaccgctaccaagagaagaatccttaaggagagaatttaccggctcactcaggcgcgacacgcactctgtcaattctccagcaaagagatccactga

SEQ ID NO: 2 - DNA, 1473 bp, homo sapiens
atgagtgaggtcaccaagaattccctggagaaaatccttccacagctgaaatgccatttcacctggaacttattcaaggaagacagtgtctcaagggatctagaagatagagtgtgtaaccagattgaatttttaaacactgagttcaaagctacaatgtacaacttgttggcctacataaaacacctagatggtaacaacgaggcagccctggaatgcttacggcaagctgaagagttaatccagcaagaacatgctgaccaagcagaaatcagaagtctagtcacttggggaaactacgcctgggtctactatcacttgggcagactctcagatgctcagatttatgtagataaggtgaaacaaacctgcaagaaattttcaaatccatacagtattgagtattctgaacttgactgtgaggaagggtggacacaactgaagtgtggaagaaatgaaagggcgaaggtgtgttttgagaaggctctggaagaaaagcccaacaacccagaattctcctctggactggcaattgcgatgtaccatctggataatcacccagagaaacagttctctactgatgttttgaagcaggccattgagctgagtcctgataaccaatacgtcaaggttctcttgggcctgaaactgcagaagatgaataaagaagctgaaggagagcagtttgttgaagaagccttggaaaagtctccttgccaaacagatgtcctccgcagtgcagccaaattttacagaagaaaaggtgacctagacaaagctattgaactgtttcaacgggtgttggaatccacaccaaacaatggctacctctatcaccagattgggtgctgctacaaggcaaaagtaagacaaatgcagaatacaggagaatctgaagctagtggaaataaagagatgattgaagcactaaagcaatatgctatggactattcgaataaagctcttgagaagggactgaatcctctgaatgcatactccgatctcgctgagttcctggagacggaatgttatcagacaccattcaataaggaagtccctgatgctgaaaagcaacaatcccatcagcgctactgcaaccttcagaaatataatgggaagtctgaagacactgctgtgcaacatggtttagagggtttgtccataagcaaaaaatcaactgacaaggaagagatcaaagaccaaccacagaatgtatctgaaaatctgcttccacaaaatgcaccaaattattggtatcttcaaggattaattcataagcagaatggagatctgctgcaagcagccaaatgttatgagaaggaactgggccgcctgctaagggatgccccttcaggcataggcagtattttcctgtcagcatctgagcttgaggatggtagtgaggaaatgggccagggcgcagtcagctccagtcccagagagctcctctctaactcagagcaactgaactga

SEQ ID NO: 3 - DNA, 378 bp, homo sapiens
atgcacaaggaggaacatgaggtggctgtgctgggggcaccccccagcaccatccttccaaggtccaccgtgatcaacatccacagcgagacctccgtgcccgaccatgtcgtctggtccctgttcaacaccctcttcttgaactggtgctgtctgggcttcatagcattcgcctactccgtgaagtctagggacaggaagatggttggcgacgtgaccggggcccaggcctatgcctccaccgccaagtgcctgaacatctgggccctgattctgggcatcctcatgaccattggattcatcctgttactggtattcggctctgtgacagtctaccatattatgttacagataatacaggaaaaacggggttactag

SEQ ID NO: 4 - DNA, 369 bp, homo sapiens
atggaggcctctgctctcacctcatcagcagtgaccagtgtggccaaagtggtcagggtggcctctggctctgccgtagttttgcccctggccaggattgctacagttgtgattggaggagttgtggccatggcggctgtgcccatggtgctcagtgccatgggcttcactgcggcgggaatcgcctcgtcctccatagcagccaagatgatgtccgcggcggccattgccaatgggggtggagttgcctcgggcagccttgtggctactctgcagtcactgggagcaactggactctccggattgaccaagttcatcctgggctccattgggtctgccattgcggctgtcattgcgaggttctactag

SEQ ID NO: 5 - DNA, 1344 bp, homo sapiens
atgcctgatttagaaaacagagtcttggatcagattgaattcctagacaccaaatacagtgtgggaatacacaacctactagcctatgtgaaacacctgaaaggccagaatgaggaagccctgaagagcttaaaagaagctgaaaacttaatgcaggaagaacatgacaaccaagcaaatgtgaggagtctggtgacctggggcaactttgcctggatgtattaccacatgggcagactggcagaagcccagacttacctggacaaggtggagaacatttgcaagaagctttcaaatcccttccgctatagaatggagtgtccagaaatagactgtgaggaaggatgggccttgctgaagtgtggaggaaagaattatgaacgggccaaggcctgctttgaaaaggtgcttgaagtggaccctgaaaacccggaatccagcgctgggtatgcgatctctgcctatcgcctggatggctttaaattagccacaaaaaatcacaagccattttctttgcttcccctaaggcaggctgtccgcttaaatccagacaatggatatattaaggttctccttgccctgaagcttcaggatgaaggacaggaagctgaaggagaaaagtacattgaagaagctctagccaacatgtcctcacagacctatgtctttcgatatgcagccaagttttaccgaagaaaaggctctgtggataaagctcttgagttattaaaaaaggccttgcaggaaacacccacttctgtcttactgcatcaccagatagggctttgctacaaggcacaaatgatccaaatcaaggaggctacaaaagggcagcctagagggcagaacagagaaaagctagacaaaatgataagatcagccatatttcattttgaatctgcagtggaaaaaaagcccacatttgaggtggctcatctagacctggcaagaatgtatatagaagcaggcaatcacagaaaagctgaagagaattttcaaaaattgttatgcatgaaaccagtggtagaagaaacaatgcaagacatacatttccactatggtcggtttcaggaatttcaaaagaaatctgacgtcaatgcaattatccattatttaaaagctataaaaatagaacaggcatcattaacaagggataaaagtatcaattctttgaagaaattggttttaaggaaacttcggagaaaggcattagatctggaaagcttgagcctccttgggttcgtctacaaattggaaggaaatatgaatgaagccctggagtactatgagcgggccctgagactggctgctgactttgagaactctgtgagacaaggtccttag

SEQ ID NO: 6 - DNA, 543 bp, homo sapiens
atggcatctacttcgtatgactattgcagagtgcccatggaagacggggataagcgctgtaagcttctgctggggataggaattctggtgctcctgatcatcgtgattctgggggtgcccttgattatcttcaccatcaaggccaacagcgaggcctgccgggacggccttcgggcagtgatggagtgtcgcaatgtcacccatctcctgcaacaagagctgaccgaggcccagaagggctttcaggatgtggaggcccaggccgccacctgcaaccacactgtgatggccctaatggcttccctggatgcagagaaggcccaaggacaaaagaaagtggaggagcttgagggagagatcactacattaaaccataagcttcaggacgcgtctgcagaggtggagcgactgagaagagaaaaccaggtcttaagcgtgagaatcgcggacaagaagtactaccccagctcccaggactccagctccgctgcggcgccccagctgctgattgtgctgctgggcctcagcgctctgctgcagtga

SEQ ID NO: 7 - DNA, 393 bp, homo sapiens
atgcggcagaaggcggtatcgcttttcttgtgctacctgctgctcttcacttgcagtggggtggaggcaggtaagaaaaagtgctcggagagctcggacagcggctccgggttctggaaggccctgaccttcatggccgtcggaggaggactcgcagtcgccgggctgcccgcgctgggcttcaccggcgccggcatcgcggccaactcggtggctgcctcgctgatgagctggtctgcgatcctgaatgggggcggcgtgcccgccggggggctagtggccacgctgcagagcctcggggctggtggcagcagcgtcgtcataggtaatattggtgccctgatgggctacgccacccacaagtatctcgatagtgaggaggatgaggagtag

SEQ ID NO: 8 - DNA, 1086 bp, homo sapiens
atgtgggtgcttacacctgctgcttttgctgggaagctcttgagtgtgttcaggcaacctctgagctctctgtggaggagcctggtcccgctgttctgctggctgagggcaaccttctggctgctagctaccaagaggagaaagcagcagctggtcctgagagggccagatgagaccaaagaggaggaagaggaccctcctctgcccaccaccccaaccagcgtcaactatcacttcactcgccagtgcaactacaaatgcggcttctgtttccacacagccaaaacatcctttgtgctgccccttgaggaagcaaagagaggattgcttttgcttaaggaagctggtatggagaagatcaacttttcaggtggagagccatttcttcaagaccggggagaatacctgggcaagttggtgaggttctgcaaagtagagttgcggctgcccagcgtgagcatcgtgagcaatggaagcctgatccgggagaggtggttccagaattatggtgagtatttggacattctcgctatctcctgtgacagctttgacgaggaagtcaatgtccttattggccgtggccaaggaaagaagaaccatgtggaaaaccttcaaaagctgaggaggtggtgtagggattatagagtcgctttcaagataaattctgtcattaatcgtttcaacgtggaagaggacatgacggaacagatcaaagcactaaaccctgtccgctggaaagtgttccagtgcctcttaattgagggtgagaattgtggagaagatgctctaagagaagcagaaagatttgttattggtgatgaagaatttgaaagattcttggagcgccacaaagaagtgtcctgcttggtgcctgaatctaaccagaagatgaaagactcctaccttattctggatgaatatatgcgctttctgaactgtagaaagggacggaaggacccttccaagtccatcctggatgttggtgtagaagaagctataaaattcagtggatttgatgaaaagatgtttctgaagcgaggaggaaaatacatatggagtaaggctgatctgaagctggattggtag

SEQ ID NO: 9 - DNA, 3078 bp, homo sapiens
atgtcgaatgggtattccacagacgagaatttccgctatctcatctcgtgcttcagggccagggtgaaaatgtacatccaggtggagcctgtgctggactacctgacctttctgcctgcagaggtgaaggagcagattcagaggacagtcgccacctccgggaacatgcaggcagttgaactgctgctgagcaccttggagaagggagtctggcaccttggttggactcgggaattcgtggaggccctccggagaaccggcagccctctggccgcccgctacatgaaccctgagctcacggacttgccctctccatcgtttgagaacgctcatgatgaatatctccaactgctgaacctccttcagcccactctggtggacaagcttctagttagagacgtcttggataagtgcatggaggaggaactgttgacaattgaagacagaaaccggattgctgctgcagaaaacaatggaaatgaatcaggtgtaagagagctactaaaaaggattgtgcagaaagaaaactggttctctgcatttctgaatgttcttcgtcaaacaggaaacaatgaacttgtccaagagttaacaggctctgattgctcagaaagcaatgcagagattgagaatttatcacaagttgatggtcctcaagtggaagagcaacttctttcaaccacagttcagccaaatctggagaaggaggtctggggcatggagaataactcatcagaatcatcttttgcagattcttctgtagtttcagaatcagacacaagtttggcagaaggaagtgtcagctgcttagatgaaagtcttggacataacagcaacatgggcagtgattcaggcaccatgggaagtgattcagatgaagagaatgtggcagcaagagcatccccggagccagaactccagctcaggccttaccaaatggaagttgcccagccagccttggaagggaagaatatcatcatctgcctccctacagggagtggaaaaaccagagtggctgtttacattgccaaggatcacttagacaagaagaaaaaagcatctgagcctggaaaagttatagttcttgtcaataaggtactgctagttgaacagctcttccgcaaggagttccaaccatttttgaagaaatggtatcgtgttattggattaagtggtgatacccaactgaaaatatcatttccagaagttgtcaagtcctgtgatattattatcagtacagctcaaatccttgaaaactccctcttaaacttggaaaatggagaagatgctggtgttcaattgtcagacttttccctcattatcattgatgaatgtcatcacaccaacaaagaagcagtgtataataacatcatgaggcattatttgatgcagaagttgaaaaacaatagactcaagaaagaaaacaaaccagtgattccccttcctcagatactgggactaacagcttcacctggtgttggaggggccacgaagcaagccaaagctgaagaacacattttaaaactatgtgccaatcttgatgcatttactattaaaactgttaaagaaaaccttgatcaactgaaaaaccaaatacaggagccatgcaagaagtttgccattgcagatgcaaccagagaagatccatttaaagagaaacttctagaaataatgacaaggattcaaacttattgtcaaatgagtccaatgtcagattttggaactcaaccctatgaacaatgggccattcaaatggaaaaaaaagctgcaaaagaaggaaatcgcaaagaacgtgtttgtgcagaacatttgaggaagtacaatgaggccctacaaattaatgacacaattcgaatgatagatgcgtatactcatcttgaaactttctataatgaagagaaagataagaagtttgcagtcatagaagatgatagtgatgagggtggtgatgatgagtattgtgatggtgatgaagatgaggatgatttaaagaaacctttgaaactggatgaaacagatagatttctcatgactttattttttgaaaacaataaaatgttgaaaaggctggctgaaaacccagaatatgaaaatgaaaagctgaccaaattaagaaataccataatggagcaatatactaggactgaggaatcagcacgaggaataatctttacaaaaacacgacagagtgcatatgcgctttcccagtggattactgaaaatgaaaaatttgctgaagtaggagtcaaagcccaccatctgattggagctggacacagcagtgagttcaaacccatgacacagaatgaacaaaaagaagtcattagtaaatttcgcactggaaaaataaatctgcttatcgctaccacagtggcagaagaaggtctggatattaaagaatgtaacattgttatccgttatggtctcgtcaccaatgaaatagccatggtccaggcccgtggtcgagccagagctgatgagagcacctacgtcctggttgctcacagtggttcaggagttatcgaacatgagacagttaatgatttccgagagaagatgatgtataaagctatacattgtgttcaaaatatgaaaccagaggagtatgctcataagattttggaattacagatgcaaagtataatggaaaagaaaatgaaaaccaagagaaatattgccaagcattacaagaataacccatcactaataactttcctttgcaaaaactgcagtgtgctagcctgttctggggaagatatccatgtaattgagaaaatgcatcacgtcaatatgaccccagaattcaaggaactttacattgtaagagaaaacaaagcactgcaaaagaagtgtgccgactatcaaataaatggtgaaatcatctgcaaatgtggccaggcttggggaacaatgatggtgcacaaaggcttagatttgccttgtctcaaaataaggaattttgtagtggttttcaaaaataattcaacaaagaaacaatacaaaaagtgggtagaattacctatcacatttcccaatcttgactattcagaatgctgtttatttagtgatgaggattag

SEQ ID NO: 10 - DNA, 1989 bp, homo sapiens
atggttgtttccgaagtggacatcgcaaaagctgatccagctgctgcatcccaccctctattactgaatggagatgctactgtggcccagaaaaatccaggctcggtggctgagaacaacctgtgcagccagtatgaggagaaggtgcgcccctgcatcgacctcattgactccctgcgggctctaggtgtggagcaggacctggccctgccagccatcgccgtcatcggggaccagagctcgggcaagagctccgtgttggaggcactgtcaggagttgcccttcccagaggcagcgggatcgtgaccagatgcccgctggtgctgaaactgaagaaacttgtgaacgaagataagtggagaggcaaggtcagttaccaggactacgagattgagatttcggatgcttcagaggtagaaaaggaaattaataaagcccagaatgccatcgccggggaaggaatgggaatcagtcatgagctaatcaccctggagatcagctcccgagatgtcccggatctgactctaatagaccttcctggcataaccagagtggctgtgggcaatcagcctgctgacattgggtataagatcaagacactcatcaagaagtacatccagaggcaggagacaatcagcctggtggtggtccccagtaatgtggacatcgccaccacagaggctctcagcatggcccaggaggtggaccccgagggagacaggaccatcggaatcttgacgaagcctgatctggtggacaaaggaactgaagacaaggttgtggacgtggtgcggaacctcgtgttccacctgaagaagggttacatgattgtcaagtgccggggccagcaggagatccaggaccagctgagcctgtccgaagccctgcagagagagaagatcttctttgagaaccacccatatttcagggatctgctggaggaaggaaaggccacggttccctgcctggcagaaaaacttaccagcgagctcatcacacatatctgtaaatctctgcccctgttagaaaatcaaatcaaggagactcaccagagaataacagaggagctacaaaagtatggtgtcgacataccggaagacgaaaatgaaaaaatgttcttcctgatagataaagttaatgcctttaatcaggacatcactgctctcatgcaaggagaggaaactgtaggggaggaagacattcggctgtttaccagactccgacacgagttccacaaatggagtacaataattgaaaacaattttcaagaaggccataaaattttgagtagaaaaatccagaaatttgaaaatcagtatcgtggtagagagctgccaggctttgtgaattacaggacatttgagacaatcgtgaaacagcaaatcaaggcactggaagagccggctgtggatatgctacacaccgtgacggatatggtccggcttgctttcacagatgtttcgataaaaaattttgaagagttttttaacctccacagaaccgccaagtccaaaattgaagacattagagcagaacaagagagagaaggtgagaagctgatccgcctccacttccagatggaacagattgtctactgccaggaccaggtatacaggggtgcattgcagaaggtcagagagaaggagctggaagaagaaaagaagaagaaatcctgggattttggggctttccaatccagctcggcaacagactcttccatggaggagatctttcagcacctgatggcctatcaccaggaggccagcaagcgcatctccagccacatccctttgatcatccagttcttcatgctccagacgtacggccagcagcttcagaaggccatgctgcagctcctgcaggacaaggacacctacagctggctcctgaaggagcggagcgacaccagcgacaagcggaagttcctgaaggagcggcttgcacggctgacgcaggctcggcgccggcttgcccagttccccggttaa

SEQ ID NO: 11 - DNA, 753 bp, homo sapiens
atgaccctgtcgccacttctgctgttcctgccaccgctgctgctgctgctggacgtccccacggcggcggtgcaggcgtcccctctgcaagcgttagacttctttgggaatgggccaccagttaactacaagacaggcaatctatacctgcgggggcccctgaagaagtccaatgcaccgcttgtcaatgtgaccctctactatgaagcactgtgcggtggctgccgagccttcctgatccgggagctcttcccaacatggctgttggtcatggagatcctcaatgtcacgctggtgccctacggaaacgcacaggaacaaaatgtcagtggcaggtgggagttcaagtgccagcatggagaagaggagtgcaaattcaacaaggtggaggcctgcgtgttggatgaacttgacatggagctagccttcctgaccattgtctgcatggaagagtttgaggacatggagagaagtctgccactatgcctgcagctctacgccccagggctgtcgccagacactatcatggagtgtgcaatgggggaccgcggcatgcagctcatgcacgccaacgcccagcggacagatgctctccagccaccgcacgagtatgtgccctgggtcaccgtcaatgggaaacccttggaagatcagacccagctccttacccttgtctgccagttgtaccagggcaagaagccggatgtctgcccttcctcaaccagctccctcaggagtgtttgcttcaagtga